European Patent Application EP 4 257 255 A1, published October 11, 2023. Title: Method for biodegrading polyolefin-derived polymers. Applicant: Consejo Superior de Investigaciones Científicas (CSIC). The sequence listing filed with the application follows.

SEQUENCE LISTING (2 sequences)

SEQ ID NO: 1 - protein, 699 aa, Galleria mellonella
MFFNLWFHCNSVTVYFLTEYFILNNLFAVDPNLVNIQKKVLLLLENWKQVDPDDEYYKIGKEYNIEANIESYTNREVVTEFLSLYKTGFTAKNQIFSIYYENQALEVRALYRLFYYAKDFETFYKTAAFARVWLNEGQFIYAFYIAVIHRADTRGIVLPAPYEIWPEYFVNSDVLAKINRIQMQKGLILPETAQYYGVLAKDNAYYFYANYSGPWTYENNENLLSYFIEDVAWNSYYYYFHSKLQFWEKGENAIGPFKERRGEIYYFIYQQILARYYLERLSNGLGEIPRFNWNDRLQAGYYPLLTTHQIPFAQRNGDYYLANDDNIEDIQFVDSYEKTFLQFLQKGQFKAYKQEVDLYNSKSVNFVGNYWQANVDLYEKVPQRNYLRSYEDAARRILGAAPRNSYENLNVPTALDFYQTSLRDPAFYQLYAKILDFINQYKEYLEPYTQDVLHFVGVKINDVKVDKLVTYFEYFDWNATNAVYLSEQQLDTGSPSYIVRQPRLNNQPFTVTIDIKSDVESEAVIKIFIGPKYDGNGYPIDLENNWVNLVEIDWFTHKLTSGQNKIERKSENFFWFKEDSVSVSKIYELLNNGQVPRYMIEKFLLLPRRLLLPRGTEGGVPFQFFVFVYPYQAPYKEWEPMKEFVVDNKPFGYPFDRPVTESYYFTQPNMYFKDVYIYQEGEEYPYYTSYWSQNQVPKH

SEQ ID NO: 2 - protein, 706 aa, Galleria mellonella
MGRLVLCVLALLVGGGISDPVKKLQRTVDQTVLDRQYKLLTLFFHPHEPIHIKEQQEIAASWDLEKNIGLYENATAVHLTIQMLHNNYQVPRGVPFTVLESVHRFEISVYYSLLYSAKTYDTFYKTAVFLRQHVNENLFVNVLSVVILHRSDTQDIRIPPIYDVFPSYFHNGEIMTTAQRITTHGQRMLEHYPSTYVWENNVVIRHNETAWPYYCNTESMPVSYFTHDVTLNALYYNIKLAYPIWLRSDACAIKEKRGELFFFWNKQLLARYYMERLSVGLGEIPELGLNEVEEGYVSGLLYHNGIPYPVRPNHLVLNHQTWHAEAIEEIEVYENRIRDMIDQGFYITNTGEHVSINSPDSIDVLGRLIEANVDSPNVQYYKDFISIWKKVLGNSLVHESVAFNGIPLVVPSVLEQYQTALRDPAYYMIMKRVLKLFNLWHEHLPHYTTKELSVPSVKIEKVEVDKLLTYFEYTNFNVTNHLHLNEIECNNVINTKSVLVQRTRLNHKVFTVRVNVKSGVAKHVTVRFFLAPKYDSVGNEIPLNVNTQNFLLIDIFNYELKEGDNLITRVSSDNLLVTDEIDSASVLFNKVDSALQGHGQYMLNMKQNILKTPRHLLLPKGRVGGMPFVLMVYISEYHAPNDVHRGTVETSTIDNTIRLTSDTLGFPVDRPLFPWMLTGVENIFLQDVQIYHKPTTEVTGVPVYVE